European Patent Specification EP 4 377 308 B1, published November 20, 2024. Title: Compounds for complexation of rare earth elements and/or s-, p-, d- block metals, their coordination compounds, peptide conjugates, method of their preparation and use thereof. Applicant: Ustav organicke chemie a biochemie AV CR, v.v.i. Application CZ. The sequence listing filed with the application follows.

SEQUENCE LISTING (29 sequences)

SEQ ID NO: 1 - protein, 6 aa, synthetic construct
  REGION 1..6: note = artificial sequence
GVHFYA

SEQ ID NO: 2 - protein, 6 aa, synthetic construct
  REGION 1..6: note = artificial sequence
RRRRRR

SEQ ID NO: 3 - protein, 7 aa, synthetic construct
  REGION 1..7: note = synthetic peptide
  SITE 1: note = X - Lutetium complex TD748, bound to the N-end of the peptidesequence via a peptide bond between -COOH group of R1 group ofTD748 (R1 is carboxyphenyl) and -NH2 group of alanine
  SITE 7: note = X - glycine amide - the C-end of the peptide sequence containsglycine, wherein the -COOH group is replaced with -C(=O)-NH2group
XAYFHVX

SEQ ID NO: 4 - protein, 7 aa, synthetic construct
  REGION 1..7: note = synthetic peptide
  SITE 1: note = X - Lutetium complex TD748, bound to the N-end of the peptidesequence via a peptide bond between -COOH group of R1 group ofTD748 (R1 is carboxyphenyl) and -NH2 group of alanine
XAYFHVG

SEQ ID NO: 5 - protein, 6 aa, synthetic construct
  REGION 1..6: note = synthetic peptide
  SITE 1: note = X - Lutetium complex TD748, bound to the N-end of the peptidesequence via a peptide bond between -COOH group of R1 group ofTD748 (R1 is carboxyphenyl) and -NH2 group of alanine
XAYFHV

SEQ ID NO: 6 - protein, 5 aa, synthetic construct
  REGION 1..5: note = synthetic peptide
  SITE 1: note = X - Lutetium complex TD748, bound to the N-end of the peptidesequence via a peptide bond between -COOH group of R1 group ofTD748 (R1 is carboxyphenyl) and -NH2 group of alanine
XAYFH

SEQ ID NO: 7 - skipped

SEQ ID NO: 8 - protein, 7 aa, synthetic construct
  REGION 1..7: note = synthetic peptide
  SITE 1: note = X - Yttrium(III) complex TD785, bound to the N-end of the peptidesequence via a peptide bond between -COOH group of R1 group ofTD785 (R1 is carboxyphenyl) and -NH2 group of alanine
  SITE 7: note = X - glycine amide - the C-end of the peptide sequence containsglycine, wherein the -COOH group is replaced with -C(=O)-NH2group
XAYFHVX

SEQ ID NO: 9 - protein, 7 aa, synthetic construct
  REGION 1..7: note = synthetic peptide
  SITE 1: note = X - Yttrium(III) complex TD785, bound to the N-end of the peptidesequence via a peptide bond between -COOH group of R1 group ofTD785 (R1 is carboxyphenyl) and -NH2 group of alanine
XAYFHVG

SEQ ID NO: 10 - protein, 6 aa, synthetic construct
  REGION 1..6: note = synthetic peptide
  SITE 1: note = X - Yttrium(III) complex TD785, bound to the N-end of the peptidesequence via a peptide bond between -COOH group of R1 group ofTD785 (R1 is carboxyphenyl) and -NH2 group of alanine
XAYFHV

SEQ ID NO: 11 - protein, 5 aa, synthetic construct
  REGION 1..5: note = synthetic peptide
  SITE 1: note = X - Yttrium(III) complex TD785, bound to the N-end of the peptidesequence via a peptide bond between -COOH group of R1 group ofTD785 (R1 is carboxyphenyl) and -NH2 group of alanine
XAYFH

SEQ ID NO: 12 - skipped

SEQ ID NO: 13 - protein, 7 aa, synthetic construct
  REGION 1..7: note = synthetic peptide
  SITE 1: note = X - Lutetium complex TD891, bound to the N-end of the peptidesequence via a peptide bond between -COOH group of R1 group ofTD891 (R1 is carboxybenzyl) and -NH2 group of alanine
  SITE 7: note = X - glycine amide - the C-end of the peptide sequence containsglycine, wherein the -COOH group is replaced with -C(=O)-NH2group
XAYFHVX

SEQ ID NO: 14 - protein, 7 aa, synthetic construct
  REGION 1..7: note = synthetic peptide
  SITE 1: note = X - Lutetium complex TD891, bound to the N-end of the peptidesequence via a peptide bond between -COOH group of R1 group ofTD891 (R1 is carboxybenzyl) and -NH2 group of alanine
XAYFHVG

SEQ ID NO: 15 - protein, 6 aa, synthetic construct
  REGION 1..6: note = synthetic peptide
  SITE 1: note = X - Lutetium complex TD891, bound to the N-end of the peptidesequence via a peptide bond between -COOH group of R1 group ofTD891 (R1 is carboxybenzyl) and -NH2 group of alanine
XAYFHV

SEQ ID NO: 16 - protein, 5 aa, synthetic construct
  REGION 1..5: note = synthetic protein
  SITE 1: note = X - Lutetium complex TD891, bound to the N-end of the peptidesequence via a peptide bond between -COOH group of R1 group ofTD891 (R1 is carboxybenzyl) and -NH2 group of alanine
XAYFH

SEQ ID NO: 17 - skipped

SEQ ID NO: 18 - protein, 7 aa, synthetic construct
  REGION 1..7: note = synthetic peptide
  SITE 1: note = X - Thulium complex TD899, bound to the N-end of the peptide sequencevia a peptide bond between -COOH group of R1 group of TD899 (R1is carboxybenzyl) and -NH2 group of alanine
  SITE 7: note = X - glycine amide - the C-end of the peptide sequence containsglycine, wherein the -COOH group is replaced with -C(=O)-NH2group
XAYFHVX

SEQ ID NO: 19 - protein, 7 aa, synthetic construct
  REGION 1..7: note = synthetic peptide
  SITE 1: note = X - Thulium complex TD899, bound to the N-end of the peptide sequencevia a peptide bond between -COOH group of R1 group of TD899 (R1is carboxybenzyl) and -NH2 group of alanine
XAYFHVG

SEQ ID NO: 20 - protein, 6 aa, synthetic construct
  REGION 1..6: note = synthetic peptide
  SITE 1: note = X - Thulium complex TD899, bound to the N-end of the peptide sequencevia a peptide bond between -COOH group of R1 group of TD899 (R1is carboxybenzyl) and -NH2 group of alanine
XAYFHV

SEQ ID NO: 21 - protein, 5 aa, synthetic construct
  REGION 1..5: note = synthetic peptide
  SITE 1: note = X - Thulium complex TD899, bound to the N-end of the peptide sequencevia a peptide bond between -COOH group of R1 group of TD899 (R1is carboxybenzyl) and -NH2 group of alanine
XAYFH

SEQ ID NO: 22 - skipped

SEQ ID NO: 23 - protein, 7 aa, synthetic construct
  REGION 1..7: note = synthetic peptide
  SITE 1: note = X - Lutetium complex TD748, bound to the N-end of the peptidesequence via a peptide bond between -COOH group of R1 group ofTD748 (R1 is carboxyphenyl) and -NH2 group of D-arginine
  SITE 2: note = D-arginine
  SITE 4: note = D-arginine
  SITE 6: note = D-arginine
  SITE 7: note = X - arginine amide - the C-end of the peptide sequence containsL-arginine, wherein the -COOH group is replaced with -C(=O)-NH2group
XRRRRRX

SEQ ID NO: 24 - protein, 7 aa, synthetic construct
  REGION 1..7: note = synthetic peptide
  SITE 1: note = X - Thulium complex TD897, bound to the N-end of the peptide sequencevia a peptide bond between -COOH group of R1 group of TD897 (R1is carboxyphenyl) and -NH2 group of D-arginine
  SITE 2: note = D-arginine
  SITE 4: note = D-arginine
  SITE 6: note = D-arginine
  SITE 7: note = X - arginine amide - the C-end of the peptide sequence containsL-arginine, wherein the -COOH group is replaced with -C(=O)-NH2group
XRRRRRX

SEQ ID NO: 25 - protein, 7 aa, synthetic construct
  REGION 1..7: note = synthetic peptide
  SITE 1: note = X - Lutetium complex TD748, bound to the N-end of the peptide sequence via a peptide bond between -COOH group of R1 group ofTD748 (R1 is carboxyphenyl) and -NH2 group of D-arginine
  SITE 2: note = D-arginine
  SITE 3: note = =NH group of L-arginine at position omega is substituted with NO2 group
  SITE 4: note = D-arginine
  SITE 5: note = =NH group of L-arginine at position omega is substituted with NO2 group
  SITE 6: note = D-arginine
  SITE 7: note = X - arginine amide - the C-end of the peptide sequence contains L-arginine, wherein the -COOH group is replaced with -C(=O)-NH2 group; and wherein =NH group at position omega is substituted with NO2 group
XRRRRRX

SEQ ID NO: 26 - protein, 7 aa, synthetic construct
  REGION 1..7: note = synthetic peptide
  SITE 1: note = X - Thulium complex TD897, bound to the N-end of the peptide sequence via a peptide bond between -COOH group of R1 group of TD748 (R1is carboxyphenyl) and -NH2 group of D-arginine
  SITE 2: note = D-arginine
  SITE 3: note = =NH group of L-arginine at position omega is substituted with NO2 group
  SITE 4: note = D-arginine
  SITE 5: note = =NH group of L-arginine at position omega is substituted with NO2 group
  SITE 6: note = D-arginine
  SITE 7: note = X - arginine amide - the C-end of the peptide sequence containsL-arginine, wherein the -COOH group is replaced with -C(=O)-NH2group; and wherein =NH group at position omega is protected withNO2 group
XRRRRRX

SEQ ID NO: 27 - protein, 6 aa, synthetic construct
  SITE 1: note = D-arginin wherein =NH group at position omega is protected with Pbf group
  SITE 2: note = L-arginin wherein =NH group at position omega is substituted with NO2 group
  SITE 3: note = D-arginin wherein =NH group at position omega is protected with Pbf group
  SITE 4: note = L-arginin wherein =NH group at position omega is substituted with NO2 group
  SITE 5: note = D-arginin wherein =NH group at position omega is protected with Pbf group
  SITE 6: note = arginine amide - the C-end of the peptide sequence contains L-arginine, wherein the -COOH group is replaced with -C(=O)-NH2 group; and wherein =NH group at position omega is substituted with NO2 group
RRRRRX

SEQ ID NO: 28 - protein, 4 aa, synthetic construct
  SITE 1: note = D-arginin wherein =NH group at position omega is protected with Pbf group
  SITE 2: note = L-arginin wherein =NH group at position omega is substituted with NO2 group
  SITE 3: note = D-arginin wherein =NH group at position omega is protected with Pbf group
  SITE 4: note = arginine amide - the C-end of the peptide sequence contains L-arginine, wherein the -COOH group is replaced with -C(=O)-NH2 group; and wherein =NH group at position omega is substituted with NO2 group
RRRR

SEQ ID NO: 29 - protein, 6 aa, synthetic construct
  SITE 1: note = D-arginin wherein =NH group at position omega is protected with Pbf group
  SITE 2: note = L-arginin wherein =NH group at position omega is protected with Pbf group
  SITE 3: note = D-arginin wherein =NH group at position omega is protected with Pbf group
  SITE 4: note = L-arginin wherein =NH group at position omega is protected with Pbf group
  SITE 5: note = D-arginin wherein =NH group at position omega is protected with Pbf group
  SITE 6: note = arginine amide - the C-end of the peptide sequence contains L-arginine, wherein the -COOH group is replaced with -C(=O)-NH2 group; and wherein =NH group at position omega is protected with Pbf group
RRRRRR